European Patent Application EP 4 464 778 A2, published November 20, 2024. Title: DIRECT OLIGONUCLEOTIDE SYNTHESIS ON CELLS AND BIOMOLECULES. Applicant: DNA SCRIPT. The sequence listing filed with the application follows.

SEQUENCE LISTING (18 sequences)

SEQ ID NO: 1 - protein, 510 aa, synthetic construct
  REGION 1..510: note = TDT enzyme
MDPLQAVHLGPRKKRPRQLGTPVASTPYDIRFRDLVLFILEKKMGTTRRAFLMELARRKGFRVENELSDSVTHIVAENNSGSDVLEWLQLQNIKASSELELLDISWLIECMGAGKPVEMMGRHQLVVNRNSSPSPVPGSQNVPAPAVKKISQYACQRRTTLNNYNQLFTDALDILAENDELRENEGSCLAFMRASSVLKSLPFPITSMKDTEGIPCLGDKVKSIIEGIIEDGESSEAKAVLNDERYKSFKLFTSVFGVGLKTAEKWFRMGFRTLSKIQSDKSLRFTQMQKAGFLYYEDLVSCVNRPEAEAVSMLVKEAVVTFLPDALVTMTGGFRRGKMTGHDVDFLITSPEATEDEEQQLLHKVTDFWKQQGLLLYCDILESTFEKFKQPSRKVDALDHFQKCFLILKLDHGRVHSEKSGQQEGKGWKAIRVDLVMCPYDRRAFALLGWTGSRQFERDLRRYATHERKMMLDNHALYDRTKRVFLEAESEEEIFAHLGLDYIEPWERNA

SEQ ID NO: 2 - protein, 381 aa, synthetic construct
  REGION 1..381: note = truncated mouse sequence
NSSPSPVPGSQNVPAPAVKKISQYACQRRTTLNNYNQLFTDALDILAENDELRENEGSCLAFMRASSVLKSLPFPITSMKDTEGIPCLGDKVKSIIEGIIEDGESSEAKAVLNDERYKSFKLFTSVFGVGLKTAEKWFRMGFRTLSKIQSDKSLRFTQMQKAGFLYYEDLVSCVNRPEAEAVSMLVKEAVVTFLPDALVTMTGGFRRGKMTGHDVDFLITSPEATEDEEQQLLHKVTDFWKQQGLLLYCDILESTFEKFKQPSRKVDALDHFQKCFLILKLDHGRVHSEKSGQQEGKGWKAIRVDLVMCPYDRRAFALLGWTGSRQFERDLRRYATHERKMMLDNHALYDRTKRVFLEAESEEEIFAHLGLDYIEPWERNA

SEQ ID NO: 3 - protein, 380 aa, synthetic construct
  REGION 1..380: note = Bovine truncated (catalytic domain):
DYSATPNPGFQKTPPLAVKKISQYACQRKTTLNNYNHIFTDAFEILAENSEFKENEVSYVTFMRAASVLKSLPFTIISMKDTEGIPCLGDKVKCIIEEIIEDGESSEVKAVLNDERYQSFKLFTSVFGVGLKTSEKWFRMGFRSLSKIMSDKTLKFTKMQKAGFLYYEDLVSCVTRAEAEAVGVLVKEAVWAFLPDAFVTMTGGFRRGKKIGHDVDFLITSPGSAEDEEQLLPKVINLWEKKGLLLYYDLVESTFEKFKLPSRQVDTLDHFQKCFLILKLHHQRVDSSKSNQQEGKTWKAIRVDLVMCPYENRAFALLGWTGSRQFERDIRRYATHERKMMLDNHALYDKTKRVFLKAESEEEIFAHLGLDYIEPWERNA

SEQ ID NO: 4 - protein, 380 aa, synthetic construct
  REGION 1..380: note = Human truncated
DYSDSTNPGPPKTPPIAVQKISQYACQRRTTLNNCNQIFTDAFDILAENCEFRENEDSCVTFMRAASVLKSLPFTIISMKDTEGIPCLGSKVKGIIEEIIEDGESSEVKAVLNDERYQSFKLFTSVFGVGLKTSEKWFRMGFRTLSKVRSDKSLKFTRMQKAGFLYYEDLVSCVTRAEAEAVSVLVKEAVWAFLPDAFVTMTGGFRRGKKMGHDVDFLITSPGSTEDEEQLLQKVMNLWEKKGLLLYYDLVESTFEKLRLPSRKVDALDHFQKCFLIFKLPRQRVDSDQSSWQEGKTWKAIRVDLVLCPYERRAFALLGWTGSRQFERDLRRYATHERKMILDNHALYDKTKRIFLKAESEEEIFAHLGLDYIEPWERNA

SEQ ID NO: 5 - protein, 376 aa, synthetic construct
  REGION 1..376: note = Chicken 1 truncated
QYPTLKTPESEVSSFTASKVSQYSCQRKTTLNNCNKKFTDAFEIMAENYEFKENEIFCLEFLRAASVLKSLPFPVTRMKDIQGLPCMGDRVRDVIEEIIEEGESSRAKDVLNDERYKSFKEFTSVFGVGVKTSEKWFRMGLRTVEEVKADKTLKLSKMQRAGFLYYEDLVSCVSKAEADAVSSIVKNTVCTFLPDALVTITGGFRRGKKIGHDIDFLITSPGQREDDELLHKGLLLYCDIIESTFVKEQIPSRHVDAMDHFQKCFAILKLYQPRVDNSSYNMSKKCDMAEVKDWKAIRVDLVITPFEQYAYALLGWTGSRQFGRDLRRYATHERKMMLDNHALYDKRKRVFLKAGSEEEIFAHLGLDYVEPWERNA

SEQ ID NO: 6 - protein, 387 aa, synthetic construct
  REGION 1..387: note = Possum truncated
SANPDPTAGTLNILPPTTKTISQYACQRRTTINNHNQRFTDAFEILAKNYEFKENDDTCLTFMRAISVLKCLPFEVVSLKDTEGLPWIGDEVKGIMEEIIEDGESLEVQAVLNDERYQSFKLFTSVFGVGLKTADKWYRMGFRTLNKIRSDKTLKLTKMQKAGLCYYEDLIDCVSKAEADAVSLLVQDAVWTFLPDALVTITGGFRRGKEFGHDVDFLITSPGAEKEQEDQLLQKVTNLWKKQGLLLYCDLIESTFEDLKLPSRKIDALDHFQKCFLILKLYHHKEDKRKWEMPTGSNESEAKSWKAIRVDLVVCPYDRYAFALLGWSGSRQFERDLRRYATHEKKMMLDNHALYDKTKKIFLKAKSEEEIFAHLGLEYIQPSERNA

SEQ ID NO: 7 - protein, 381 aa, synthetic construct
  REGION 1..381: note = New truncated shrew
DCPASHDSSPQKTESAAVQKISQYACQRRTTLNNHNHIFTDAFEILAENCEFRENEGSYVTYMRAASVLKSLPFSIISMKDTEGIPCLADKVKCVIEEIIEDGESSEVKAVLNDERYKSFKLFTSVFGVGLKTAEKWFRLGFRTLSGIMNDKTLKLTHMQKAGFLYYEDLVSCVTRAEAEAVGVLVKEAVWAFLPDAIVTMTGGFRRGKKVGHDVDFLITSPEATEEQEQQLLHKVITFWEKEGLLLYCDLYESTFEKLKMPSRKVDALDHFQKCFLILKLHRECVDDGTSSQLQGKTWKAIRVDLVVCPYECRAFALLGWTGSPQFERDLRRYATHERKMMLDNHALYDKTKRKFLSADSEEDIFAHLGLDYIEPWERNA

SEQ ID NO: 8 - protein, 387 aa, synthetic construct
  REGION 1..387: note = Python truncated
EKYQLPEDEDRSVTSDLDRDSISEYACQRRTTLKNYNQKFTDAFEILAENYEFNENKGFCTAFRRAASVLKCLPFTIVQVHDIEGVPWMGKQVKGIIEDIIEEGESSKVKAVLDNENYRSVKLFTSVFGVGLKTSDKWYRMGLRTLEEVKRDKNLKLTRMQKAGFLHYDDLTSCVSKAEADAASLIVQDVVWKIVPNAIVTIAGGFRRGKQTGHDVDFLITVPGSKQEEEELLHTVIDIWKKQELLLYYDLIESTFEDTKLPSRKVDALDHFQKCFAILKVHKEREDKGNSIRSKAFSEEEIKDWKAIRVDLVVVPFEQYAFALLGWTGSTQFERDLRRYATHEKKMMLDNHALYDKTKKIFLNAASEEEIFAHLGLDYLEPWERNA

SEQ ID NO: 9 - protein, 381 aa, synthetic construct
  REGION 1..381: note = truncated dog
DYTASPNPELQKTLPVAVKKISQYACQRRTTLNNYNNVFTDAFEVLAENYEFRENEVFSLTFMRAASVLKSLPFTIISMKDTEGIPCLGDQVKCIIEEIIEDGESSEVKAVLNDERYQSFKLFTSVFGVGLKTSEKWFRMGFRTLSKIKSDKSLKFTPMQKAGFLYYEDLVSCVTRAEAEAVGVLVKEAVGAFLPDAFVTMTGGFRRGKKMGHDVDFLITSPGSTDEDEEQLLPKVINLWERKGLLLYCDLVESTFEKLKLPSRKVDALDHFQKCFLILKLHHQRVDGGKCSQQEGKTWKAIRVDLVMCPYERRAFALLGWTGSRQFERDLRRYASHERKMILDNHALYDKTKKIFLKAESEEEIFAHLGLDYIEPWERNA

SEQ ID NO: 10 - protein, 382 aa, synthetic construct
  REGION 1..382: note = TRUNC MOLE
GDCPASHDSSPQKTESAAVQKISQYACQRRTTLNNHNHIFTDAFEILAENCEFRENEGSYVTYMRAASVLKSLPFSIISMKDTEGIPCLADKVKCVIEEIIEDGESSEVKAVLNDERYKSFKLFTSVFGVGLKTAEKWFRLGFRTLSGIMNDKTLKLTHMQKAGFLYYEDLVSCVTRAEAEAVGVLVKEAVWAFLPDAIVTMTGGFRRGKKVGHDVDFLITSPEATEEQEQQLLHKVITFWEKEGLLLYCDLYESTFEKLKMPSRKVDALDHFQKCFLILKLHRECVDDGTSSQLQGKTWKAIRVDLVVCPYECRAFALLGWTGSPQFERDLRRYATHERKMMLDNHALYDKTKRKFLSADSEEDIFAHLGLDYIEPWERNA

SEQ ID NO: 11 - protein, 379 aa, synthetic construct
  REGION 1..379: note = Pika trunk
EYSANPSPGPQATPAVYKISQYACQRRTTLNNHNHIFTDAFEILAENYEFKENEGCYVTYMRAASVLKSLPFTIVSMKDTEGIPCLEDKVKSIMEEIIEEGESSEVKAVLSDERYQCFKLFTSVFGVGLKTSEKWFRMGFRSLSNIRLDKSLKFTQMQKAGFRYYEDIVSCVTRAEAEAVDVLVNEAVRAFLPDAFITMTGGFRRGKKIGHDVDFLITSPELTEEDEQQLLHKVMNLWEKKGLLLYHDLVESTFEKLKQPSRKVDALDHFQKCFLIFKLYHERVGGDRCRQPEGKDWKAIRVDLVMCPYECHAFALLGWTGSRQFERDLRRYASHERKMILDNHALYDKTKRVFLQAENEEEIFAHLGLDYIEPWERNA

SEQ ID NO: 12 - protein, 384 aa, synthetic construct
  REGION 1..384: note = TRUNC HEDGEHOG
DASFGSNPGSQNTPPLAIKKISQYACQRRTSLNNCNHIFTDALDILAENHEFRENEVSCVAFMRAASVLKSLPFTIISMKDTKGIPCLGDKAKCVIEEIIEDGESSEVKAILNDERYQSFKLFTSVFGVGLKTSEKWFRMGFRTLNKIMSDKTLKLTRMQKAGFLYYEDLVSCVAKAEADAVSVLVQEAVWAFLPDAMVTMTGGFRRGKKLGHDVDFLITSPGATEEEEQQLLPKVINFWERKGLLLYHDLVESTFEKLKLPSRKVDALDHFQKCFLILKLHLQHVNGVGNSKTGQQEGKNWKAIRVDLVMCPYERRAFALLGWTGSRQFERDLRRFATHERKMMLDNHALYDKTKRIFLKAESEEEIFAHLGLDYIDPWERNA

SEQ ID NO: 13 - protein, 381 aa, synthetic construct
  REGION 1..381: note = truncated tree shrew
DHSTSPSPGPQKTPALAVQKISQYACQRRTTLNNCNRVFTDAFETLAENYEFRENEDSSVIFLRAASVLRSLPFTITSMRDTEGLPCLGDKVKCVIEEIIEDGESSEVNAVLNDERYKSFKLFTSVFGVGLKTSEKWFRMGFRTLSRVRSDKSLHLTRMQQAGFLYYEDLASCVTRAEAEAVGVLVKEAVGAFLPDALVTITGGFRRGKKTGHDVDFLITSPGSTEEKEEELLQKVLNLWEKKGLLLYYDLVESTFEKLKTPSRKVDALDHFPKCFLILKLHHQRVDGDKPSQQEGKSWKAIRVDLVMCPYERHAFALLGWTGSRQFERDLRRYATHERKMMLDNHALYDKTKRVFLKAESEEDIFAHLGLDYIEPWERNA

SEQ ID NO: 14 - protein, 394 aa, synthetic construct
  REGION 1..394: note = TRUNCATED PLATYPUS
LTNSAPINCMTETPSLATKQVSQYACERRTTLNNCNQKFTDAFEILAKDFEFRENEGICLAFMRAISVLKCLPFTIVRMKDIEGVPWLGDQVKSIIEEIIEDGESSSVKAVLNDERYRSFQLFNSVFEVGLTDNGENGIARGFQTLNEVITDENISLTKTTLSTSLWNYLPGFLYYEDLVSCVAKEEADAVYLIVKEAVRAFLPEALVTLTGGFRRGKKIGHDVDFLISDPESGQDEQLLPNIIKLWEKQELLLYYDLVESTFEKTKIPSRKVDAMDHFQKCFLILKLHHQKVDSGRYKPPPESKNHEAKNWKAIRVDLVMCPFEQYAYALLGWTGSRQFERDLRRYATHEKKMMLDNHALYDKTKKIFLKAESEEDIFTHLGLDYIEPWERNA

SEQ ID NO: 15 - protein, 384 aa, synthetic construct
  REGION 1..384: note = TRUNCATED JERBOA
SSELELLDVSWLIECMGAGKPVEMTGRHQLVKQTFCLPGFILQDAFDILAENCEFRENEASCVEFMRAASVLKSLPFPIISVKDTEGIPWLGGKVKCVIEEIIEDGESSEVKALLNDERYKSFKLFTSVFGVGLKTAERWFRMGFRTLSTVKLDKSLTFTRMQKAGFLHYEDLVSCVTRAEAEAVSVLVQQAVVAFLPDALVSMTGGFRRGKKIGHDVDFLITSPEATEEEEQQLLHKVTNFWEQKGLLLYCDHVESTFEKCKLPSRKVDALDHFQKCFLILKLYRERVDSVKSSQQEGKGWKAIRVDLVMCPYECRAFALLGWTGSRQFERDLRRYATHERKMRLDNHALYDKTKRVFLKAESEEEIFAHLGLEYIEPLERNA

SEQ ID NO: 16 - skipped

SEQ ID NO: 17 - DNA, 15 bp, synthetic construct
  misc_feature 1..15: note = Exemplary cDNA produced in process of Fig. 4A
  misc_feature 15: note = n is a, c, g, t or u
  source 1..15: mol_type = other DNA
ttttttttttttttn

SEQ ID NO: 18 - skipped